European Patent Specification EP 4 211 269 B1, published November 6, 2024. Title: COMPOSITIONS AND METHODS FOR AMPLIFYING POLYNUCLEOTIDES. Applicant: ILLUMINA, INC. ILLUMINA CAMBRIDGE LIMITED. The sequence listing filed with the application follows.

SEQUENCE LISTING (8 sequences)

SEQ ID NO: 1 - DNA, 20 bp, Artificial Sequence
  source: /note="Description of Artificial Sequence: Synthetic primer"
aatgatacggcgaccaccga

SEQ ID NO: 2 - DNA, 21 bp, Artificial Sequence
  source: /note="Description of Artificial Sequence: Synthetic primer"
caagcagaagacggcatacga

SEQ ID NO: 3 - DNA, 21 bp, Artificial Sequence
  source: /note="Description of Artificial Sequence: Synthetic primer"
ttttttcaagcagaagacggc

SEQ ID NO: 4 - DNA, 21 bp, Artificial Sequence
  source: /note="Description of Artificial Sequence: Synthetic primer"
tttttaatgatacggcgacca

SEQ ID NO: 5 - DNA, 20 bp, Artificial Sequence
  source: /note="Description of Artificial Sequence: Synthetic oligonucleotide"
tcggtggtcgccgtatcatt

SEQ ID NO: 6 - DNA, 20 bp, Artificial Sequence
  source: /note="Description of Artificial Sequence: Synthetic oligonucleotide"
cacatctagagccaccagcg

SEQ ID NO: 7 - DNA, 21 bp, Artificial Sequence
  source: /note="Description of Artificial Sequence: Synthetic oligonucleotide"
tcgtatgccgtcttctgcttg

SEQ ID NO: 8 - DNA, 15 bp, Artificial Sequence
  source: /note="Description of Artificial Sequence: Synthetic oligonucleotide"
tagagcatacggcag